European Patent Application EP 4 796 623 A1, published August 26, 2026. Title: YEAST STRAINS AND USES THEREOF. Applicant: Danstar Ferment AG. The sequence listing filed with the application follows.

SEQUENCE LISTING (5 sequences)

SEQ ID NO: 1 - DNA, 2421 bp, Saccharomyces cerevisiae
  source 1..2421: mol_type = genomic DNA
  CDS 1..2421: protein_id = 2; translation = MQRPFLLAYLVLSLLFNSALGFPTALVPRGSSSSNITSSGPSSTPFSSATESFSTGTTVTPSSSKYPGSKTETSVSSTTETTIVPTTTTTSVITPSTTTITTTVCSTGTNSAGETTSGCSPKTITTTVPCSTSPSETASESTTTSPTTPVTTVVSTTVVTTEYSTSTKQGGEITTTFVTKNIPTTYLTTIAPTSSVTTVTNFTPTTITTTVCSTGTNSAGETTSGCSPKTVTTTVPCSTGTGEYTTEATAPVTTAVTTTVVTTESSTGTNSAGKTTTSYTTKSVPTTYVFDFGKGILDQSCGGVFSNNGSSQVQLRDAVLMNGTVVYDSNGAWDSSALEEWLQRQKKVSIERIFENIGPSAVYPSILPGVVIASPSQTHPDYFYQWIRDSALTINSIVSHSADPAIETLLQYLNVSFHLQRTNNTLGAGIGYTNDTVALGDPKWNVDNTAFTEPWGRPQNDGPALRSIAILKIIDYIKQSGTDLGAKYPFQSTADIFDDIVRWDLRFIIDHWNSSGFDLWEEVNGMHFFTLLVQLSAVDRSLSYFNASERSSPFVEELRQTRRDISKFLVDPANGFINGKYNYIVETPMIADTLRSGLDISTLLAANTVHDAPSASHLPFDINDPAVLNTLHHLMLHMRSIYPINDSSKNATGIALGRYPEDVYDGYGVGEGNPWVLATCAASTTLYQLIYRHISEQHDLVVPMNNDCSNAFWSELVFSNLTTLGNDEGYLILEFNTPAFNQTIQKIFQLADSFLVKLKAHVGTDGELSEQFNKYTGFMQGAQHLTWSYTSFWDAYQIRQEVLQSL
atgcaaagaccatttctactcgcttatttggtcctttcgcttctatttaactcagctttgggttttccaactgcactagttcctagaggatcctcctctagcaacatcacttcctccggtccatcttcaactccattcagctctgctactgaaagcttttctactggcactactgtcactccatcatcatccaaataccctggcagtaaaacagaaacttctgtttcttctacaaccgaaactaccattgttccaactacaactacgacttctgtcataacaccatcaacaaccactattaccactacggtttgctctacaggaacaaactctgccggtgaaactacttctggatgctctccaaagaccattacaactactgttccatgttcaaccagtccaagcgaaaccgcatcggaatcaacaaccacttcacctaccacacctgtaactacagttgtctcaaccaccgtcgttactactgagtattctactagtacaaaacaaggtggtgaaattacaactacatttgtcaccaaaaacattccaaccacttacctaactacaattgctccaacttcatcagtcactacggttaccaatttcaccccaaccactattactactacggtttgctctacaggaacaaactctgccggtgaaactacctctggatgctctccaaagactgtcacaacaactgttccttgttcaactggtactggcgaatacactactgaagctaccgcccctgttacaacagctgtcacaaccaccgttgttaccactgaatcctctacgggtactaactccgctggtaagacgacaactagttacacaacaaagtctgtaccaaccacctatgtatttgactttggcaagggcattctcgatcaaagctgcggcggtgtattttcaaacaacggctcttcgcaagtgcagctgcgggatgcagtcttgatgaatgggacagtggtatacgattcaaacggcgcttgggacagtagtgcgctggaggagtggctccagcgacagaaaaaagtttccatcgaaagaatatttgaaaatattgggcccagcgccgtgtatccgtctattttgcctggggtcgtgattgcgtcaccatcgcaaacgcatccagactacttctaccaatggataagggacagcgcgttgacgataaacagtattgtctctcattctgcggacccggcaatagagacgttattgcagtacctgaacgtttcattccacttgcaaagaaccaacaacacattgggcgctggcattggttacactaacgatacagtggctttgggagaccctaagtggaacgtcgacaacacggctttcacggaaccttggggtcgtcctcaaaacgatggccctgctcttcgaagcattgccatcttaaaaatcatcgactacatcaagcaatctggcactgatctgggggccaagtacccattccagtccaccgcagatatctttgatgatattgtacgttgggacctgaggttcattattgaccactggaattcttccggatttgatctatgggaggaagtcaatggcatgcatttctttactttactggtacaactgtctgcagtggacaggtcgctgtcgtattttaacgcctcagaacggtcgtctccctttgttgaagaattgcgtcagacacgccgggacatctccaagtttttagtggaccctgcgaatgggtttatcaacggcaagtacaattatattgttgagacacccatgattgccgacacattgagatccggactggacatatccactttattagctgcgaacaccgtccacgatgcgccatctgcttcccatcttccgttcgatatcaatgaccctgccgtcctgaacacgttgcaccatttgatgttgcacatgcgttcgatataccccatcaacgatagctccaaaaatgcaacgggtattgccctgggccggtatcctgaggacgtatatgatggatatggcgttggcgagggaaatccctgggtcctggccacgtgtgccgcttcaacaacgctttatcagctcatttacagacacatctctgagcagcatgacttggttgtcccaatgaacaacgattgttcgaacgcattttggagcgagctggtattctccaacctcacgactttgggaaatgacgaaggctatttgattttggagttcaatacacctgccttcaatcaaaccatacaaaaaatcttccaactagctgattcattcttggtcaagctgaaagctcacgtgggaacagacggggaactaagtgaacaatttaacaaatacacagggtttatgcagggtgcccaacaccttacctggtcctatacttcattctgggatgcctatcaaataagacaagaagttttacagagtttgtag

SEQ ID NO: 2 - protein, 806 aa, Saccharomyces cerevisiae
MQRPFLLAYLVLSLLFNSALGFPTALVPRGSSSSNITSSGPSSTPFSSATESFSTGTTVTPSSSKYPGSKTETSVSSTTETTIVPTTTTTSVITPSTTTITTTVCSTGTNSAGETTSGCSPKTITTTVPCSTSPSETASESTTTSPTTPVTTVVSTTVVTTEYSTSTKQGGEITTTFVTKNIPTTYLTTIAPTSSVTTVTNFTPTTITTTVCSTGTNSAGETTSGCSPKTVTTTVPCSTGTGEYTTEATAPVTTAVTTTVVTTESSTGTNSAGKTTTSYTTKSVPTTYVFDFGKGILDQSCGGVFSNNGSSQVQLRDAVLMNGTVVYDSNGAWDSSALEEWLQRQKKVSIERIFENIGPSAVYPSILPGVVIASPSQTHPDYFYQWIRDSALTINSIVSHSADPAIETLLQYLNVSFHLQRTNNTLGAGIGYTNDTVALGDPKWNVDNTAFTEPWGRPQNDGPALRSIAILKIIDYIKQSGTDLGAKYPFQSTADIFDDIVRWDLRFIIDHWNSSGFDLWEEVNGMHFFTLLVQLSAVDRSLSYFNASERSSPFVEELRQTRRDISKFLVDPANGFINGKYNYIVETPMIADTLRSGLDISTLLAANTVHDAPSASHLPFDINDPAVLNTLHHLMLHMRSIYPINDSSKNATGIALGRYPEDVYDGYGVGEGNPWVLATCAASTTLYQLIYRHISEQHDLVVPMNNDCSNAFWSELVFSNLTTLGNDEGYLILEFNTPAFNQTIQKIFQLADSFLVKLKAHVGTDGELSEQFNKYTGFMQGAQHLTWSYTSFWDAYQIRQEVLQSL

SEQ ID NO: 3 - DNA, 2451 bp, Saccharomyces cerevisiae
  source 1..2451: mol_type = genomic DNA
tagtacttgctttattccgtgtatcgtactttaggtcgtcagttttacacttcggtacgcaaatgaaaataaaaagctcattcacaacttagacacaatttcgccatttacaagtagctgaagagtccatctatcgaattatgaatgatgctattttaaatatcgtcgttgctgcactcgttttccatgttctttttatccacacatccgatgttttatttacagttgagcatctcagggccagcgacaaatataaacatattatactcaaaatgaagctcgttgaaaagaggatatttcttaacctcttttacagtgttttcaacaccttttcatctgtgtgccatgtcagattaaggatgctcaacttttcgaattattattacaaatttcaaagaaattactattcctttttgtcccctaatgtatccctcatttcataccgtcgttttggggttccaactgcacatagctttcaagtgtggttttacggtaagaacaacccccccatcggttggtgcggaatactttcctattctcatcgagagccgagccatacacctaaggtggacagaaagctaaaattccaaaacagaaaaatctaacatctttgctcccttacaagtaggaacgctagcgtatcaacccatctccagatttgcccagcatttctgtagaacacccaatgcgaatgaagactaatgaatattttaaagacaaaaaataggaaaagtttaattattgatggttctcaccaccgcaaaacggtcacttgcatgcattgaggacatgcatctgcagtacttgtttttctcgaatgttttttaccatctcttttttccttatctgagctgctgacgcagacggacattgtttcatatttcgaaagctgtgcgggaaaacggaccctaacacgaatgtggatgcgctaatcggtatttccacctcatgaaacctgctactttttcagtgctcttcgtatgcatttcccaaaattcattcgtagccttgtcaacttagactcagttccacggcgtgcaggacggggtattatgaataaaggatccacgggtaagatttgttctatgttttaggtatggagttttgtaccacaaaactttaggaataccggattgtgtgcctacgccagccccagagtatgttctcacggctgtaattcctagtgatcttttcctggctcaaattaaactttcgcggcaggaaaaaaaaggctttttcttttttgtgtttcagtttctcggaatgtggcattacataagcataatcctttttgggtgtgcctggaaagttcaaattaagggttttttcttctgttttcttgacaagaaaatgttgcccaaagagtttcggccgttattttcctatcgaagtgggtcctttttgtctttagtccttctctggggctagcgatcgctgcaaaattaggcttcactggtacgagttaactttttttctttttttttgtcatccttttctttggggctaagaatggacttcccttttctttttctttgttgcagcagtggcttcaaagaactgctgattgctcaaggcaatcagttaaaagaaaaattagctttttttgtcaggcattgcacaaacttttttatttctgcctatactcttagacagatcagtcattcatgttgtctttttaacggtcgtactgggacatcgcataccttgagattccgtaattaggtgcaacaatacgggcacaactcattctgcggtatcttcacggacagaatttctattgcctattggtggtgtgattaacaattggaagcgcagagcttagaatggattttcaattcaatggatttggaggtattcgtttgtttactaatatttactttgaggacattgcccaaccctaaaagtgcctgttccagaacagaataacattatgatacgttttcctgaccgctgagcaatttaaagcaattagtagggtacgattgtttctagagaaatgtgggtcatctttttaggtccgttctcttctgatgaggtaacctttacaaaaatgtcatggagttaccaattgggattcaaggcatcatcacaatatacttcgttcttttacggagaaattaagctctttctactttgaattaactgttagacttgtcttatctgagaaatgtccgtgttcaaattaaataaaaatttagggcagttttatttaccttaacaaatatgttcaagcatttacgttactgcgctctcttctagttcaagaacggataactcatagacttacctgtacaagttgttgaagggttctcaattgataaaaaaggatcttttgcttcctaaactaaacctataaaaagcaccctattcatcagttataatctcttgtcatgttgtggttctaattgaaaatatactatggtaggcctcaaaaatccatatacgcacact

SEQ ID NO: 4 - DNA, 4872 bp, Saccharomyces cerevisiae
  source 1..4872: mol_type = genomic DNA
tagtacttgctttattccgtgtatcgtactttaggtcgtcagttttacacttcggtacgcaaatgaaaataaaaagctcattcacaacttagacacaatttcgccatttacaagtagctgaagagtccatctatcgaattatgaatgatgctattttaaatatcgtcgttgctgcactcgttttccatgttctttttatccacacatccgatgttttatttacagttgagcatctcagggccagcgacaaatataaacatattatactcaaaatgaagctcgttgaaaagaggatatttcttaacctcttttacagtgttttcaacaccttttcatctgtgtgccatgtcagattaaggatgctcaacttttcgaattattattacaaatttcaaagaaattactattcctttttgtcccctaatgtatccctcatttcataccgtcgttttggggttccaactgcacatagctttcaagtgtggttttacggtaagaacaacccccccatcggttggtgcggaatactttcctattctcatcgagagccgagccatacacctaaggtggacagaaagctaaaattccaaaacagaaaaatctaacatctttgctcccttacaagtaggaacgctagcgtatcaacccatctccagatttgcccagcatttctgtagaacacccaatgcgaatgaagactaatgaatattttaaagacaaaaaataggaaaagtttaattattgatggttctcaccaccgcaaaacggtcacttgcatgcattgaggacatgcatctgcagtacttgtttttctcgaatgttttttaccatctcttttttccttatctgagctgctgacgcagacggacattgtttcatatttcgaaagctgtgcgggaaaacggaccctaacacgaatgtggatgcgctaatcggtatttccacctcatgaaacctgctactttttcagtgctcttcgtatgcatttcccaaaattcattcgtagccttgtcaacttagactcagttccacggcgtgcaggacggggtattatgaataaaggatccacgggtaagatttgttctatgttttaggtatggagttttgtaccacaaaactttaggaataccggattgtgtgcctacgccagccccagagtatgttctcacggctgtaattcctagtgatcttttcctggctcaaattaaactttcgcggcaggaaaaaaaaggctttttcttttttgtgtttcagtttctcggaatgtggcattacataagcataatcctttttgggtgtgcctggaaagttcaaattaagggttttttcttctgttttcttgacaagaaaatgttgcccaaagagtttcggccgttattttcctatcgaagtgggtcctttttgtctttagtccttctctggggctagcgatcgctgcaaaattaggcttcactggtacgagttaactttttttctttttttttgtcatccttttctttggggctaagaatggacttcccttttctttttctttgttgcagcagtggcttcaaagaactgctgattgctcaaggcaatcagttaaaagaaaaattagctttttttgtcaggcattgcacaaacttttttatttctgcctatactcttagacagatcagtcattcatgttgtctttttaacggtcgtactgggacatcgcataccttgagattccgtaattaggtgcaacaatacgggcacaactcattctgcggtatcttcacggacagaatttctattgcctattggtggtgtgattaacaattggaagcgcagagcttagaatggattttcaattcaatggatttggaggtattcgtttgtttactaatatttactttgaggacattgcccaaccctaaaagtgcctgttccagaacagaataacattatgatacgttttcctgaccgctgagcaatttaaagcaattagtagggtacgattgtttctagagaaatgtgggtcatctttttaggtccgttctcttctgatgaggtaacctttacaaaaatgtcatggagttaccaattgggattcaaggcatcatcacaatatacttcgttcttttacggagaaattaagctctttctactttgaattaactgttagacttgtcttatctgagaaatgtccgtgttcaaattaaataaaaatttagggcagttttatttaccttaacaaatatgttcaagcatttacgttactgcgctctcttctagttcaagaacggataactcatagacttacctgtacaagttgttgaagggttctcaattgataaaaaaggatcttttgcttcctaaactaaacctataaaaagcaccctattcatcagttataatctcttgtcatgttgtggttctaattgaaaatatactatggtaggcctcaaaaatccatatacgcacactatgcaaagaccatttctactcgcttatttggtcctttcgcttctatttaactcagctttgggttttccaactgcactagttcctagaggatcctcctctagcaacatcacttcctccggtccatcttcaactccattcagctctgctactgaaagcttttctactggcactactgtcactccatcatcatccaaataccctggcagtaaaacagaaacttctgtttcttctacaaccgaaactaccattgttccaactacaactacgacttctgtcataacaccatcaacaaccactattaccactacggtttgctctacaggaacaaactctgccggtgaaactacttctggatgctctccaaagaccattacaactactgttccatgttcaaccagtccaagcgaaaccgcatcggaatcaacaaccacttcacctaccacacctgtaactacagttgtctcaaccaccgtcgttactactgagtattctactagtacaaaacaaggtggtgaaattacaactacatttgtcaccaaaaacattccaaccacttacctaactacaattgctccaacttcatcagtcactacggttaccaatttcaccccaaccactattactactacggtttgctctacaggaacaaactctgccggtgaaactacctctggatgctctccaaagactgtcacaacaactgttccttgttcaactggtactggcgaatacactactgaagctaccgcccctgttacaacagctgtcacaaccaccgttgttaccactgaatcctctacgggtactaactccgctggtaagacgacaactagttacacaacaaagtctgtaccaaccacctatgtatttgactttggcaagggcattctcgatcaaagctgcggcggtgtattttcaaacaacggctcttcgcaagtgcagctgcgggatgcagtcttgatgaatgggacagtggtatacgattcaaacggcgcttgggacagtagtgcgctggaggagtggctccagcgacagaaaaaagtttccatcgaaagaatatttgaaaatattgggcccagcgccgtgtatccgtctattttgcctggggtcgtgattgcgtcaccatcgcaaacgcatccagactacttctaccaatggataagggacagcgcgttgacgataaacagtattgtctctcattctgcggacccggcaatagagacgttattgcagtacctgaacgtttcattccacttgcaaagaaccaacaacacattgggcgctggcattggttacactaacgatacagtggctttgggagaccctaagtggaacgtcgacaacacggctttcacggaaccttggggtcgtcctcaaaacgatggccctgctcttcgaagcattgccatcttaaaaatcatcgactacatcaagcaatctggcactgatctgggggccaagtacccattccagtccaccgcagatatctttgatgatattgtacgttgggacctgaggttcattattgaccactggaattcttccggatttgatctatgggaggaagtcaatggcatgcatttctttactttactggtacaactgtctgcagtggacaggtcgctgtcgtattttaacgcctcagaacggtcgtctccctttgttgaagaattgcgtcagacacgccgggacatctccaagtttttagtggaccctgcgaatgggtttatcaacggcaagtacaattatattgttgagacacccatgattgccgacacattgagatccggactggacatatccactttattagctgcgaacaccgtccacgatgcgccatctgcttcccatcttccgttcgatatcaatgaccctgccgtcctgaacacgttgcaccatttgatgttgcacatgcgttcgatataccccatcaacgatagctccaaaaatgcaacgggtattgccctgggccggtatcctgaggacgtatatgatggatatggcgttggcgagggaaatccctgggtcctggccacgtgtgccgcttcaacaacgctttatcagctcatttacagacacatctctgagcagcatgacttggttgtcccaatgaacaacgattgttcgaacgcattttggagcgagctggtattctccaacctcacgactttgggaaatgacgaaggctatttgattttggagttcaatacacctgccttcaatcaaaccatacaaaaaatcttccaactagctgattcattcttggtcaagctgaaagctcacgtgggaacagacggggaactaagtgaacaatttaacaaatacacagggtttatgcagggtgcccaacaccttacctggtcctatacttcattctgggatgcctatcaaataagacaagaagttttacagagtttgtag

SEQ ID NO: 5 - DNA, 5124 bp, Saccharomyces cerevisiae
  source 1..5124: mol_type = genomic DNA
tagtacttgctttattccgtgtatcgtactttaggtcgtcagttttacacttcggtacgcaaatgaaaataaaaagctcattcacaacttagacacaatttcgccatttacaagtagctgaagagtccatctatcgaattatgaatgatgctattttaaatatcgtcgttgctgcactcgttttccatgttctttttatccacacatccgatgttttatttacagttgagcatctcagggccagcgacaaatataaacatattatactcaaaatgaagctcgttgaaaagaggatatttcttaacctcttttacagtgttttcaacaccttttcatctgtgtgccatgtcagattaaggatgctcaacttttcgaattattattacaaatttcaaagaaattactattcctttttgtcccctaatgtatccctcatttcataccgtcgttttggggttccaactgcacatagctttcaagtgtggttttacggtaagaacaacccccccatcggttggtgcggaatactttcctattctcatcgagagccgagccatacacctaaggtggacagaaagctaaaattccaaaacagaaaaatctaacatctttgctcccttacaagtaggaacgctagcgtatcaacccatctccagatttgcccagcatttctgtagaacacccaatgcgaatgaagactaatgaatattttaaagacaaaaaataggaaaagtttaattattgatggttctcaccaccgcaaaacggtcacttgcatgcattgaggacatgcatctgcagtacttgtttttctcgaatgttttttaccatctcttttttccttatctgagctgctgacgcagacggacattgtttcatatttcgaaagctgtgcgggaaaacggaccctaacacgaatgtggatgcgctaatcggtatttccacctcatgaaacctgctactttttcagtgctcttcgtatgcatttcccaaaattcattcgtagccttgtcaacttagactcagttccacggcgtgcaggacggggtattatgaataaaggatccacgggtaagatttgttctatgttttaggtatggagttttgtaccacaaaactttaggaataccggattgtgtgcctacgccagccccagagtatgttctcacggctgtaattcctagtgatcttttcctggctcaaattaaactttcgcggcaggaaaaaaaaggctttttcttttttgtgtttcagtttctcggaatgtggcattacataagcataatcctttttgggtgtgcctggaaagttcaaattaagggttttttcttctgttttcttgacaagaaaatgttgcccaaagagtttcggccgttattttcctatcgaagtgggtcctttttgtctttagtccttctctggggctagcgatcgctgcaaaattaggcttcactggtacgagttaactttttttctttttttttgtcatccttttctttggggctaagaatggacttcccttttctttttctttgttgcagcagtggcttcaaagaactgctgattgctcaaggcaatcagttaaaagaaaaattagctttttttgtcaggcattgcacaaacttttttatttctgcctatactcttagacagatcagtcattcatgttgtctttttaacggtcgtactgggacatcgcataccttgagattccgtaattaggtgcaacaatacgggcacaactcattctgcggtatcttcacggacagaatttctattgcctattggtggtgtgattaacaattggaagcgcagagcttagaatggattttcaattcaatggatttggaggtattcgtttgtttactaatatttactttgaggacattgcccaaccctaaaagtgcctgttccagaacagaataacattatgatacgttttcctgaccgctgagcaatttaaagcaattagtagggtacgattgtttctagagaaatgtgggtcatctttttaggtccgttctcttctgatgaggtaacctttacaaaaatgtcatggagttaccaattgggattcaaggcatcatcacaatatacttcgttcttttacggagaaattaagctctttctactttgaattaactgttagacttgtcttatctgagaaatgtccgtgttcaaattaaataaaaatttagggcagttttatttaccttaacaaatatgttcaagcatttacgttactgcgctctcttctagttcaagaacggataactcatagacttacctgtacaagttgttgaagggttctcaattgataaaaaaggatcttttgcttcctaaactaaacctataaaaagcaccctattcatcagttataatctcttgtcatgttgtggttctaattgaaaatatactatggtaggcctcaaaaatccatatacgcacactatgcaaagaccatttctactcgcttatttggtcctttcgcttctatttaactcagctttgggttttccaactgcactagttcctagaggatcctcctctagcaacatcacttcctccggtccatcttcaactccattcagctctgctactgaaagcttttctactggcactactgtcactccatcatcatccaaataccctggcagtaaaacagaaacttctgtttcttctacaaccgaaactaccattgttccaactacaactacgacttctgtcataacaccatcaacaaccactattaccactacggtttgctctacaggaacaaactctgccggtgaaactacttctggatgctctccaaagaccattacaactactgttccatgttcaaccagtccaagcgaaaccgcatcggaatcaacaaccacttcacctaccacacctgtaactacagttgtctcaaccaccgtcgttactactgagtattctactagtacaaaacaaggtggtgaaattacaactacatttgtcaccaaaaacattccaaccacttacctaactacaattgctccaacttcatcagtcactacggttaccaatttcaccccaaccactattactactacggtttgctctacaggaacaaactctgccggtgaaactacctctggatgctctccaaagactgtcacaacaactgttccttgttcaactggtactggcgaatacactactgaagctaccgcccctgttacaacagctgtcacaaccaccgttgttaccactgaatcctctacgggtactaactccgctggtaagacgacaactagttacacaacaaagtctgtaccaaccacctatgtatttgactttggcaagggcattctcgatcaaagctgcggcggtgtattttcaaacaacggctcttcgcaagtgcagctgcgggatgcagtcttgatgaatgggacagtggtatacgattcaaacggcgcttgggacagtagtgcgctggaggagtggctccagcgacagaaaaaagtttccatcgaaagaatatttgaaaatattgggcccagcgccgtgtatccgtctattttgcctggggtcgtgattgcgtcaccatcgcaaacgcatccagactacttctaccaatggataagggacagcgcgttgacgataaacagtattgtctctcattctgcggacccggcaatagagacgttattgcagtacctgaacgtttcattccacttgcaaagaaccaacaacacattgggcgctggcattggttacactaacgatacagtggctttgggagaccctaagtggaacgtcgacaacacggctttcacggaaccttggggtcgtcctcaaaacgatggccctgctcttcgaagcattgccatcttaaaaatcatcgactacatcaagcaatctggcactgatctgggggccaagtacccattccagtccaccgcagatatctttgatgatattgtacgttgggacctgaggttcattattgaccactggaattcttccggatttgatctatgggaggaagtcaatggcatgcatttctttactttactggtacaactgtctgcagtggacaggtcgctgtcgtattttaacgcctcagaacggtcgtctccctttgttgaagaattgcgtcagacacgccgggacatctccaagtttttagtggaccctgcgaatgggtttatcaacggcaagtacaattatattgttgagacacccatgattgccgacacattgagatccggactggacatatccactttattagctgcgaacaccgtccacgatgcgccatctgcttcccatcttccgttcgatatcaatgaccctgccgtcctgaacacgttgcaccatttgatgttgcacatgcgttcgatataccccatcaacgatagctccaaaaatgcaacgggtattgccctgggccggtatcctgaggacgtatatgatggatatggcgttggcgagggaaatccctgggtcctggccacgtgtgccgcttcaacaacgctttatcagctcatttacagacacatctctgagcagcatgacttggttgtcccaatgaacaacgattgttcgaacgcattttggagcgagctggtattctccaacctcacgactttgggaaatgacgaaggctatttgattttggagttcaatacacctgccttcaatcaaaccatacaaaaaatcttccaactagctgattcattcttggtcaagctgaaagctcacgtgggaacagacggggaactaagtgaacaatttaacaaatacacagggtttatgcagggtgcccaacaccttacctggtcctatacttcattctgggatgcctatcaaataagacaagaagttttacagagtttgtagacaaaaaaaaataaaagaaaagcgagaagtatacacaagtgtatttcctagatatttacatcaaatatatatatatatacttatttacaaaactctgatattataaattaattagatactatgtcggaacgtccagcccaaccacgtttgcagttcttttcactttctcatcctgtgtcaacttgttgccaggattgtatctgtcgaccagctcctcgtattctctttggttgtccaaggacttgatgatgc